European Patent Specification EP 3 472 347 B1, published January 4, 2023. Title: IN VITRO NEPHROTOXICITY SCREENING ASSAY. Applicant: F. Hoffmann la Roche AG. The sequence listing filed with the application follows.

SEQUENCE LISTING (20 sequences)

SEQ ID NO: 1 - DNA, 16 bp, Artificial
  Oligonucleotide motif
cgtcagtatgcgaatc

SEQ ID NO: 2 - DNA, 16 bp, Artificial
  Oligonucleotide motif
aatgctacaaaaccca

SEQ ID NO: 3 - DNA, 14 bp, Artificial
  Oligonucleotide motif
tgctacaaaaccca

SEQ ID NO: 4 - DNA, 15 bp, Artificial
  Oligonucleotide motif
gctgtgtgagcttgg

SEQ ID NO: 5 - DNA, 16 bp, Artificial
  Oligonucleotide motif
taaggcaatcaaggta

SEQ ID NO: 6 - DNA, 16 bp, Artificial
  Oligonucleotide motif
caaaggaaacacacat

SEQ ID NO: 7 - DNA, 16 bp, Artificial
  Oligonucleotide motif
caaatgctgaaactat

SEQ ID NO: 8 - DNA, 16 bp, Artificial
  Oligonucleotide motif
actgctttccactctg

SEQ ID NO: 9 - DNA, 16 bp, Artificial
  Oligonucleotide motif
gcctcccagttccttt

SEQ ID NO: 10 - DNA, 16 bp, Artificial
  Oligonucleotide motif
cacattccttgctctg

SEQ ID NO: 11 - DNA, 14 bp, Artificial
  Oligonucleotide motif
tgctcaacatcaag

SEQ ID NO: 12 - DNA, 14 bp, Artificial
  Oligonucleotide motif
ttacacttgaccca

SEQ ID NO: 13 - DNA, 14 bp, Artificial
  Oligonucleotide motif
tttacacttgaccc

SEQ ID NO: 14 - DNA, 16 bp, Artificial
  Oligonucleotide motif
gtcagaaacaaccacc

SEQ ID NO: 15 - DNA, 14 bp, Artificial
  Oligonucleotide motif
ctatgtgttcctgt

SEQ ID NO: 16 - DNA, 16 bp, Artificial
  Oligonucleotide motif
cgtttgtgctcgataa

SEQ ID NO: 17 - DNA, 15 bp, Artificial
  Oligonucleotide motif
cgtttgtgctcgata

SEQ ID NO: 18 - DNA, 16 bp, Artificial
  Oligonucleotide motif
attgcattgtttccgt

SEQ ID NO: 19 - DNA, 16 bp, Artificial
  Oligonucleotide motif
cattgcattgtttccg

SEQ ID NO: 20 - DNA, 12 bp, Artificial
  Oligonucleotide motif
ggcatgagcttc